European Patent Application EP 4 461 145 A1, published November 13, 2024. Title: LACTIC ACID BACTERIAL STRAIN, COMPOSITION FOR IMPROVING GUT MICROBIOTA COMPOSITION, PRODUCT OF SAID LACTIC ACID BACTERIAL STRAIN, AND METHOD FOR THE PREPARATION OF THE COMPOSITION THEREOF. Applicant: SUNWAY BIOTECH CO., LTD. Application EP. The sequence listing filed with the application follows.

SEQUENCE LISTING (6 sequences)

SEQ ID NO: 1 - DNA, 22 bp, Artificial sequence
  source 1..22: mol_type = other DNA
ttgtggtggagtaagggtagtg

SEQ ID NO: 2 - DNA, 21 bp, Artificial sequence
  source 1..21: mol_type = other DNA
agacggcacaaacatggatac

SEQ ID NO: 3 - DNA, 20 bp, Artificial sequence
  source 1..20: mol_type = other DNA
tgaatgcgcagagacaaacg

SEQ ID NO: 4 - DNA, 21 bp, Artificial sequence
  source 1..21: mol_type = other DNA
ggtggccatttcaagtagtcc

SEQ ID NO: 5 - DNA, 115 bp, Pediococcus acidilactici
  source 1..115: mol_type = other DNA
ttgtggtggagtaagggtagtggcaattgacagagaaaattgtatacaaaagttgttaattctatttttattaaattttaaccatttagtttatgtatccatgtttgtgccgtct

SEQ ID NO: 6 - DNA, 505 bp, Pediococcus acidilactici
  source 1..505: mol_type = other DNA
tgaatgcgcagagacaaacgctagagtctcgaatcgaggcaaaaaaattgactaaaagtgaaacaaaaaaagtgagaattgaaagcacaaaatctgttggtaggaaagcctcaatggatctattgaaccaaagctggggggatatgattgttgatatcattggtgcacatgaagagattgagggaaagcttaatgagtctaaagaagctcttttacttggggagtatttaaataaatcagataaccaggaatatgcgttaaaacggcttattaatgtaattaccgatccgtatggcagcatcttatttaataaactgcttttaatattaaaagattatccggctgatggggacatgatggatatcttaagagatacattattaaacttgtccgatgtaaataactttaaaagtgtttttacaaagtacaaatttctaatctcactaattgataggataacccctcaggctatggtaattttacaggactacttgaaatggccacc